European Patent Specification EP 3 701 024 B1, published April 22, 2026. Title: VECTORS. Applicant: Autolus Limited. The sequence listing filed with the application follows.

SEQUENCE LISTING (47 sequences)

SEQ ID NO: 1 - protein, 202 aa, Escherichia coli
MKALTARQQEVFDLIRDHISQTGMPPTRAEIAQRLGFRSPNAAEEHLKALARKGVIEIVSGASRGIRLLQEEEEGLPLVGRVAAGEPLLAQQHIEGHYQVDPSLFKPNADFLLRVSGMSMKDIGIMDGDLLAVHKTQDVRNGQVVVARIDDEVTVKRLKKQGNKVELLPENSEFKPIVVDLRQQSFTIEGLAVGVIRNGDWL

SEQ ID NO: 2 - protein, 363 aa, Escherichia coli
MVNVKPVTLYDVAEYAGVSYQTVSRVVNQASHVSAKTREKVEAAMAELNYIPNRVAQQLAGKQSLLIGVATSSLALHAPSQIVAAIKSRADQLGASVVVSMVERSGVEACKAAVHNLLAQRVSGLIINYPLDDQDAIAVEAACTNVPALFLDVSDQTPINSIIFSHEDGTRLGVEHLVALGHQQIALLAGPLSSVSARLRLAGWHKYLTRNQIQPIAEREGDWSAMSGFQQTMQMLNEGIVPTAMLVANDQMALGAMRAITESGLRVGADISVVGYDDTEDSSCYIPPLTTIKQDFRLLGQTSVDRLLQLSQGQAVKGNQLLPVSLVKRKTTLAPNTQTASPRALADSLMQLARQVSRLESGQ

SEQ ID NO: 3 - protein, 208 aa, Escherichia coli
MMSRLDKSKVINSALELLNEVGIEGLTTRKLAQKLGVEQPTLYWHVKNKRALLDALAIEMLDRHHTHFCPLEGESWQDFLRNNAKSFRCALLSHRDGAKVHLGTRPTEKQYETLENQLAFLCQQGFSLENALYALSAVGHFTLGCVLEDQEHQVAKEERETPTTDSMPPLLRQAIELFDHQGAEPAFLFGLELIICGLEKQLKCESGS

SEQ ID NO: 4 - protein, 881 aa, Saccharomyces cerevisiae
MKLLSSIEQACDICRLKKLKCSKEKPKCAKCLKNNWECRYSPKTKRSPLTRAHLTEVESRLERLEQLFLLIFPREDLDMILKMDSLQDIKALLTGLFVQDNVNKDAVTDRLASVETDMPLTLRQHRISATSSSEESSNKGQRQLTVSIDSAAHHDNSTIPLDFMPRDALHGFDWSEEDDMSDGLPFLKTDPNNNGFFGDGSLLCILRSIGFKPENYTNSNVNRLPTMITDRYTLASRSTTSRLLQSYLNNFHPYCPIVHSPTLMMLYNNQIEIASKDQWQILFNCILAIGAWCIEGESTDIDVFYYQNAKSHLTSKVFESGSIILVTALHLLSRYTQWRQKTNTSYNFHSFSIRMAISLGLNRDLPSSFSDSSILEQRRRIWWSVYSWEIQLSLLYGRSIQLSQNTISFPSSVDDVQRTTTGPTIYHGIIETARLLQVFTKIYELDKTVTAEKSPICAKKCLMICNEIEEVSRQAPKFLQMDISTTALTNLLKEHPWLSFTRFELKWKQLSLIIYVLRDFFTNFTQKKSQLEQDQNDHQSYEVKRCSIMLSDAAQRTVMSVSSYMDNHNVTPYFAWNCSYYLFNAVLVPIKTLLSNSKSNAENNETAQLLQQINTVLMLLKKLATFKIQTCEKYIQVLEEVCAPFLLSQCAIPLPHISYNNSNGSAIKNIVGSATIAQYPTLPEENVNNISVKYVSPGSVGPSPVPLKSGASFSDLVKLLSNRPPSRNSPVTIPRSTPSHRSVTPFLGQQQQLQSLVPLTPSALFGGANFNQSGNIADSSLSFTFTNSSNGPNLITTQTNSQALSQPIASSNVHDNFMNNEITASKIDDGNNSKPLSPGWTDQTAYNAFGITTGMFNTTTMDDVYNYLFDDEDTPPNPKKE

SEQ ID NO: 5 - protein, 816 aa, Neurospora crassa
MPPKRKTLNAAAEANAHADGHADGNADGHVANTAASSNNARFADLTNIDTPGLGPTTTTLLVEPARSKRQRVSRACDQCRAAREKCDGIQPACFPCVSQGRSCTYQASPKKRGVQTGYIRTLELALAWMFENVARSEDALHNLLVRDAGQGSALLVGKDSPAAERLHARWATSRVNKSITRLLSGQAAQDPSEDGQSPSEDINVQDAGAKTSDFPHAPHLTFSAPKSSTAETRTLPGPVRPPISANTLENNLQPDGTGIGKLPPNHWRLLDIYFSYTHSWLPILEKKDMYQALYQYSEQGSLLPSANVESGVHAELWSALALASFQAAATAASSATGPASAAHGHDNAINPSPADISDTARKLIPLESGPFQVQHCRALLLLCLVSLGRDDWESAWLLVGFAVRVLLVVRTQLPPDDDRPRPRMRALLVACFIVDTIVSMRHNVPAHLKPDDIADLPLPEDGQDQWEPWTPCEGLGGEHTMLQMLRNPAYPLSTFNHLYGVTKLVALELLPRIRTSSQNAPLEFRSRLQQVIGHNSPFSVFVLSQDTASAFVPTAYLTRTVYLWAAAFSEPLNEHYSHLLIETLDQYQKRFGTYAIPPLIPSLLDSLLALKKQSHSSERHRRHLEELFPAYSSIWPRGGRHSNTGLQPIRQLELPPTATATASIMPHVMEQPLSTSINPVNDRFNGIPNPTPYNSDAALDAITQTNDYGSVNTHGILSTYPPPATHLNEASVALAPGGAPPRPPPPYVDSTTNHPPYHSNLVPMANFGYSTVDYDAMVDDLASIEYTDAVDVDPQFMTNLGFVPGCNFSDISTYEQ

SEQ ID NO: 6 - protein, 93 aa, herpes simplex virus
EFPGIRRPAGIPGDLAPPTDVSLGDELHLDGEDVAMAHADALDDFDLDMLGDGDSPGPGFTPHDSAPYGALDMADFEFEQMFTDALGIDEYGG

SEQ ID NO: 7 - protein, 295 aa, Artificial Sequence
  amino acid sequence of LexA/VP16 fusion
MKALTARQQEVFDLIRDHISQTGMPPTRAEIAQRLGFRSPNAAEEHLKALARKGVIEIVSGASRGIRLLQEEEEGLPLVGRVAAGEPLLAQQHIEGHYQVDPSLFKPNADFLLRVSGMSMKDIGIMDGDLLAVHKTQDVRNGQVVVARIDDEVTVKRLKKQGNKVELLPENSEFKPIVVDLRQQSFTIEGLAVGVIRNGDWLEFPGIRRPAGIPGDLAPPTDVSLGDELHLDGEDVAMAHADALDDFDLDMLGDGDSPGPGFTPHDSAPYGALDMADFEFEQMFTDALGIDEYGG

SEQ ID NO: 8 - protein, 436 aa, Artificial Sequence
  amino acid sequence of lactose repressor/VP16 fusion
MVNVKPVTLYDVAEYAGVSYQTVSRVVNQASHVSAKTREKVEAAMAELNYIPNRVAQQLAGKQSLLIGVATSSLALHAPSQIVAAIKSRADQLGASVVVSMVERSGVEACKAAVHNLLAQRVSGLIINYPLDDQDAIAVEAACTNVPALFLDVSDQTPINSIIFSHEDGTRLGVEHLVALGHQQIALLAGPLSSVSARLRLAGWHKYLTRNQIQPIAEREGDWSAMSGFQQTMQMLNEGIVPTAMLVANDQMALGAMRAITESGLRVGADISVVGYDDTEDSSCYIPPLTTIKQDFRLLGQTSVDRLLQLSQGQAVKGNQLLPVSLVKRKTTLAPNTQTASPRALADSLMQLARQVSRAPPTDVSLGDELHLDGEDVAMAHADALDDFDLDMLGDGDSPGPGFTPHDSAPYGALDMADFEFEQMFTDALGIDEYGG

SEQ ID NO: 9 - protein, 336 aa, Artificial Sequence
  amino acid sequence of tetracycline-controlled transactivator (tTA)
MMSRLDKSKVINSALELLNEVGIEGLTTRKLAQKLGVEQPTLYWHVKNKRALLDALAIEMLDRHHTHFCPLEGESWQDFLRNNAKSFRCALLSHRDGAKVHLGTRPTEKQYETLENQLAFLCQQGFSLENALYALSAVGHFTLGCVLEDQEHQVAKEERETPTTDSMPPLLRQAIELFDHQGAEPAFLFGLELIICGLEKQLKCESGSAYSRARTKNNYGSTIEGLLDLPDDDAPEEAGLAAPRLSFLPAGHTRRLSTAPPTDVSLGDELHLDGEDVAMAHADALDDFDLDMLGDGDSPGPGFTPHDSAPYGALDMADFEFEQMFTDALGIDEYGG

SEQ ID NO: 10 - protein, 232 aa, Artificial Sequence
  amino acid sequence of GAL4/VP16 fusion protein
MKLLSSIEQACDICRLKKLKCSKEKPKCAKCLKNNWECRYSPKTKRSPLTRAHLTEVESRLERLEQLFLLIFPREDLDMILKMDSLQDIKALLTGLFVQDNVNKDAVTDRLASVETDMPLTLRQHRISATSSSEESSNKGQRQLTVSPEFPGIWAPPTDVSLGDELHLDGEDVAMAHADALDDFDLDMLGDGDSPGPGFTPHDSAPYGALDMADFEFEQMFTDALGIDEYGG

SEQ ID NO: 11 - protein, 382 aa, Artificial Sequence
  amino acid sequence of LexA/QF fusion protein
MPPKKKRKVEDPMKALTARQQEVFDLIRDHISQTGMPPTRAEIAQRLGFRSPNAAEEHLKALARKGVIEIVSGASRGIRLLQEEEEGLPLVGRVAAGEPLLAQQHIEGHYQVDPSLFKPNADFLLRVSGMSMKDIGIMDGDLLAVHKTQDVRNGQVVVARIDDEVTVKRLKKQGNKVELLPENSEFKPIVVDLRQQSFTIEGLAVGVIRNGDWLGRQLELPPTATATASIMPHVMEQPLSTSINPVNDRFNGIPNPTPYNSDAALDAITQTNDYGSVNTHGILSTYPPPATHLNEASVALAPGGAPPRPPPPYVDSTTNHPPYHSNLVPMANFGYSTVDYDAMVDDLASIEYTDAVDVDPQFMTNLGFVPGCNFSDINTYEQ

SEQ ID NO: 12 - DNA, 8 bp, Artificial Sequence
  DNA binding sequence of Brain-1
atttgcat

SEQ ID NO: 13 - protein, 500 aa, Homo sapiens
MATAASNPYLPGNSLLAAGSIVHSDAAGAGGGGGGGGGGGGGGAGGGGGGMQPGSAAVTSGAYRGDPSSVKMVQSDFMQGAMAASNGGHMLSHAHQWVTALPHAAAAAAAAAAAAVEASSPWSGSAVGMAGSPQQPPQPPPPPPQGPDVKGGAGRDDLHAGTALHHRGPPHLGPPPPPPHQGHPGGWGAAAAAAAAAAAAAAAAHLPSMAGGQQPPPQSLLYSQPGGFTVNGMLSAPPGPGGGGGGAGGGAQSLVHPGLVRGDTPELAEHHHHHHHHAHPHPPHPHHAQGPPHHGGGGGGAGPGLNSHDPHSDEDTPTSDDLEQFAKQFKQRRIKLGFTQADVGLALGTLYGNVFSQTTICRFEALQLSFKNMCKLKPLLNKWLEEADSSTGSPTSIDKIAAQGRKRKKRTSIEVSVKGALESHFLKCPKPSAQEITNLADSLQLEKEVVRVWFCNRRQKEKRMTPPGIQQQTPDDVYSQVGTVSADTPPPHHGLQTSVQ

SEQ ID NO: 14 - protein, 443 aa, Homo sapiens
MATAASNHYSLLTSSASIVHAEPPGGMQQGAGGYREAQSLVQGDYGALQSNGHPLSHAHQWITALSHGGGGGGGGGGGGGGGGGGGGGDGSPWSTSPLGQPDIKPSVVVQQGGRGDELHGPGALQQQHQQQQQQQQQQQQQQQQQQQQQRPPHLVHHAANHHPGPGAWRSAAAAAHLPPSMGASNGGLLYSQPSFTVNGMLGAGGQPAGLHHHGLRDAHDEPHHADHHPHPHSHPHQQPPPPPPPQGPPGHPGAHHDPHSDEDTPTSDDLEQFAKQFKQRRIKLGFTQADVGLALGTLYGNVFSQTTICRFEALQLSFKNMCKLKPLLNKWLEEADSSSGSPTSIDKIAAQGRKRKKRTSIEVSVKGALESHFLKCPKPSAQEITSLADSLQLEKEVVRVWFCNRRQKEKRMTPPGGTLPGAEDVYGGSRDTPPHHGVQTPVQ

SEQ ID NO: 15 - DNA, 15 bp, Artificial Sequence
  DNA binding site of NFIC
  misc_feature (6)..(10): n is a, c, g, or t
ttggcnnnnngccaa

SEQ ID NO: 16 - protein, 508 aa, Homo sapiens
MYSSPLCLTQDEFHPFIEALLPHVRAFAYTWFNLQARKRKYFKKHEKRMSKDEERAVKDELLGEKPEVKQKWASRLLAKLRKDIRPECREDFVLSITGKKAPGCVLSNPDQKGKMRRIDCLRQADKVWRLDLVMVILFKGIPLESTDGERLVKAAQCGHPVLCVQPHHIGVAVKELDLYLAYFVRERDAEQSGSPRTGMGSDQEDSKPITLDTTDFQESFVTSGVFSVTELIQVSRTPVVTGTGPNFSLGELQGHLAYDLNPASTGLRRTLPSTSSSGSKRHKSGSMEEDVDTSPGGDYYTSPSSPTSSSRNWTEDMEGGISSPVKKTEMDKSPFNSPSPQDSPRLSSFTQHHRPVIAVHSGIARSPHPSSALHFPTTSILPQTASTYFPHTAIRYPPHLNPQDPLKDLVSLACDPASQQPGPLNGSGQLKMPSHCLSAQMLAPPPPGLPRLALPPATKPATTSEGGATSPTSPSYSPPDTSPANRSFVGLGPRDPAGIYQAQSWYLG

SEQ ID NO: 17 - DNA, 15 bp, Artificial Sequence
  DNA binding site of NFIC
  misc_feature (6)..(10): n is a, c, g, or t
ttggcnnnnngccaa

SEQ ID NO: 18 - protein, 502 aa, Homo sapiens
MYSPYCLTQDEFHPFIEALLPHVRAFSYTWFNLQARKRKYFKKHEKRMSKDEERAVKDELLGEKPEIKQKWASRLLAKLRKDIRPEFREDFVLTITGKKPPCCVLSNPDQKGKIRRIDCLRQADKVWRLDLVMVILFKGIPLESTDGERLYKSPQCSNPGLCVQPHHIGVTIKELDLYLAYFVHTPESGQSDSSNQQGDADIKPLPNGHLSFQDCFVTSGVWNVTELVRVSQTPVATASGPNFSLADLESPSYYNINQVTLGRRSITSPPSTSTTKRPKSIDDSEMESPVDDVFYPGTGRSPAAGSSQSSGWPNDVDAGPASLKKSGKLDFCSALSSQGSSPRMAFTHHPLPVLAGVRPGSPRATASALHFPSTSIIQQSSPYFTHPTIRYHHHHGQDSLKEFVQFVCSDGSGQATGQPNGSGQGKVPGSFLLPPPPPVARPVPLPMPDSKSTSTAPDGAALTPPSPSFATTGASSANRFVSIGPRDGNFLNIPQQSQSWFL

SEQ ID NO: 19 - DNA, 6 bp, Artificial Sequence
  DNA binding site of MyoD
  misc_feature (3)..(4): n is a, c, g, or t
canntg

SEQ ID NO: 20 - protein, 320 aa, Homo sapiens
MELLSPPLRDVDLTAPDGSLCSFATTDDFYDDPCFDSPDLRFFEDLDPRLMHVGALLKPEEHSHFPAAVHPAPGAREDEHVRAPSGHHQAGRCLLWACKACKRKTTNADRRKAATMRERRRLSKVNEAFETLKRCTSSNPNQRLPKVEILRNAIRYIEGLQALLRDQDAAPPGAAAAFYAPGPLPPGRGGEHYSGDSDASSPRSNCSDGMMDYSGPPSGARRRNCYEGAYYNEAPSEPRPGKSAAVSSLDCLSSIVERISTESPAAPALLLADVPSESPPRRQEAAAPSEGESSGDPTQSPDAAPQCPAGANPNPIYQVL

SEQ ID NO: 21 - DNA, 10 bp, Artificial Sequence
  DNA binding site of MEF2A
ytawwwwtar

SEQ ID NO: 22 - protein, 506 aa, Homo sapiens
MGRKKIQITRIMDERNRQVTFTKRKFGLMKKAYELSVLCDCEIALIIFNSSNKLFQYASTDMDKVLLKYTEYNEPHESRTNSDIVEALNKKEHRGCDSPDPDTSYVLTPHTEEKYKKINEEFDNMMRNHKIAPGLPPQNFSMSVTVPVTSPNALSYTNPGSSLVSPSLAASSTLTDSSMLSPPQTTLHRNVSPGAPQRPPSTGNAGGMLSTTDLTVPNGAGSSPVGNGFVNSRASPNLIGATGANSLGKVMPTKSPPPPGGGNLGMNSRKPDLRVVIPPSSKGMMPPLSEEEELELNTQRISSSQATQPLATPVVSVTTPSLPPQGLVYSAMPTAYNTDYSLTSADLSALQGFNSPGMLSLGQVSAWQQHHLGQAALSSLVAGGQLSQGSNLSINTNQNISIKSEPISPPRDRMTPSGFQQQQQQQQQQQPPPPPQPQPQPPQPQPRQEMGRSPVDSLSSSSSSYDGSDREDPRGDFHSPIVLGRPPNTEDRESPSVKRMRMDAWV

SEQ ID NO: 23 - DNA, 7 bp, Artificial Sequence
  DNA-binding site of KLF3
cmcaccc

SEQ ID NO: 24 - protein, 345 aa, Homo sapiens
MLMFDPVPVKQEAMDPVSVSYPSNYMESMKPNKYGVIYSTPLPEKFFQTPEGLSHGIQMEPVDLTVNKRSSPPSAGNSPSSLKFPSSHRRASPGLSMPSSSPPIKKYSPPSPGVQPFGVPLSMPPVMAAALSRHGIRSPGILPVIQPVVVQPVPFMYTSHLQQPLMVSLSEEMENSSSSMQVPVIESYEKPISQKKIKIEPGIEPQRTDYYPEEMSPPLMNSVSPPQALLQENHPSVIVQPGKRPLPVESPDTQRKRRIHRCDYDGCNKVYTKSSHLKAHRRTHTGEKPYKCTWEGCTWKFARSDELTRHFRKHTGIKPFQCPDCDRSFSRSDHLALHRKRHMLV

SEQ ID NO: 25 - protein, 1437 aa, Artificial Sequence
  amino acid sequence of dCas9/VP64
MKKKRKVEASDKKYSIGLAIGTNSVGWAVITDEYKVPSKKFKVLGNTDRHSIKKNLIGALLFDSGETAEATRLKRTARRRYTRRKNRICYLQEIFSNEMAKVDDSFFHRLEESFLVEEDKKHERHPIFGNIVDEVAYHEKYPTIYHLRKKLVDSTDKADLRLIYLALAHMIKFRGHFLIEGDLNPDNSDVDKLFIQLVQTYNQLFEENPINASGVDAKAILSARLSKSRRLENLIAQLPGEKKNGLFGNLIALSLGLTPNFKSNFDLAEDAKLQLSKDTYDDDLDNLLAQIGDQYADLFLAAKNLSDAILLSDILRVNTEITKAPLSASMIKRYDEHHQDLTLLKALVRQQLPEKYKEIFFDQSKNGYAGYIDGGASQEEFYKFIKPILEKMDGTEELLVKLNREDLLRKQRTFDNGSIPHQIHLGELHAILRRQEDFYPFLKDNREKIEKILTFRIPYYVGPLARGNSRFAWMTRKSEETITPWNFEEVVDKGASAQSFIERMTNFDKNLPNEKVLPKHSLLYEYFTVYNELTKVKYVTEGMRKPAFLSGEQKKAIVDLLFKTNRKVTVKQLKEDYFKKIECFDSVEISGVEDRFNASLGTYHDLLKIIKDKDFLDNEENEDILEDIVLTLTLFEDREMIEERLKTYAHLFDDKVMKQLKRRRYTGWGRLSRKLINGIRDKQSGKTILDFLKSDGFANRNFMQLIHDDSLTFKEDIQKAQVSGQGDSLHEHIANLAGSPAIKKGILQTVKVVDELVKVMGRHKPENIVIEMARENQTTQKGQKNSRERMKRIEEGIKELGSQILKEHPVENTQLQNEKLYLYYLQNGRDMYVDQELDINRLSDYDVDAIVPQSFLKDDSIDNKVLTRSDKNRGKSDNVPSEEVVKKMKNYWRQLLNAKLITQRKFDNLTKAERGGLSELDKAGFIKRQLVETRQITKHVAQILDSRMNTKYDENDKLIREVKVITLKSKLVSDFRKDFQFYKVREINNYHHAHDAYLNAVVGTALIKKYPKLESEFVYGDYKVYDVRKMIAKSEQEIGKATAKYFFYSNIMNFFKTEITLANGEIRKRPLIETNGETGEIVWDKGRDFATVRKVLSMPQVNIVKKTEVQTGGFSKESILPKRNSDKLIARKKDWDPKKYGGFDSPTVAYSVLVVAKVEKGKSKKLKSVKELLGITIMERSSFEKNPIDFLEAKGYKEVKKDLIIKLPKYSLFELENGRKRMLASAGELQKGNELALPSKYVNFLYLASHYEKLKGSPEDNEQKQLFVEQHKHYLDEIIEQISEFSKRVILADANLDKVLSAYNKHRDKPIREQAENIIHLFTLTNLGAPAAFKYFDTTIDRKRYTSTKEVLDATLIHQSITGLYETRIDLSQLGGDPKKKRKVDALDDFDLDMLGSDALDDFDLDMLGSDALDDFDLDMLGSDALDDFDLDMLYID

SEQ ID NO: 26 - DNA, 103 bp, Artificial Sequence
  5-repeat GAL4 upstream activating sequence
cggagtactgtcctccgagcggagtactgtcctccgactcgagcggagtactgtcctccgatcggagtactgtcctccgcgaattccggagtactgtcctccg

SEQ ID NO: 27 - DNA, 271 bp, Artificial Sequence
  Tet response element (TRE)
tccctatcagtgatagagaaaagtgaaagtcgagtttaccactccctatcagtgatagagaaaagtgaaagtcgagtttaccactccctatcagtgatagagaaaagtgaaagtcgagtttaccactccctatcagtgatagagaaaagtgaaagtcgagtttaccactccctatcagtgatagagaaaagtgaaagtcgagtttaccactccctatcagtgatagagaaaagtgaaagtcgagtttaccactccctatcagtgatagaga

SEQ ID NO: 28 - DNA, 78 bp, Artificial Sequence
  LacI promoter sequence
gacaccatcgaatggcgcaaaacctttcgcggtatggcatgatagcgcccggaagagagtcaattcagggtggtgaat

SEQ ID NO: 29 - DNA, 257 bp, Mus musculus
ggtctgaaaaggatttggagaaggggagctgaattcatttgcttttgtctgttaccagctctgggggcagagagagagccatcccctgggaacagcctgagaattcccacttcccctgaggagccctcccttcttaggccctccagatggtagtgtggacaaaaggcaataattagcatgagaatcggcctccctcccagaggatgaggtcatcggccttggccttgggtggggaggcggagactgatctgaggagt

SEQ ID NO: 30 - DNA, 507 bp, Artificial Sequence
  Glial Fibrillary Acidic Protein (GFAP) promoter sequence
acatatcctggtgtggagtaggggacgctgctctgacagaggctcgggggcctgagctggctctgtgagctggggaggaggcagacagccaggccttgtctgcaagcagacctggcagcattgggctggccgccccccagggcctcctcttcatgcccagtgaatgactcaccttggcacagacacaatgttcggggtgggcacagtgcctgcttcccgccgcaccccagcccccctcaaatgccttccgagaagcccattgagcagggagctctccccatagctgggctgcggcccaaccccaccccctcaggctatgccagggggtgttgccaggggcacccgggcatcgccagtctagcccactccttcataaagccctcgcatcccaggagcgagcagagccagagcaggttggagaggagacgcatcacctccgctgctcgcggggatcctctagagtcgacggatccggggaattccccagtctcaggatccaccatgggg

SEQ ID NO: 31 - DNA, 151 bp, Mus musculus
atccactggaaacgtcttgatgtgcagcaacagcttagaggggggctcaggtttctgtggcgttggctatatttatctctgggttcatgccagcagggagggtttaaatggcacccagcagttggtgtgaggggctgcgggagcttggggg

SEQ ID NO: 32 - DNA, 142 bp, Mus musculus
ccactacgggtctaggctgcccatgtaaggaggcaaggcctggggacacccgagatgcctggttataattaacccagacatgtggctgcccccccccccccaacacctgctgcctctaaaaataaccctgtccctggtggat

SEQ ID NO: 33 - DNA, 771 bp, Artificial Sequence
  Murine muscle creatine kinase/alpha-myosin heavy chain (MHCK7) promoter
ccttcagattaaaaataactgaggtaagggcctgggtaggggaggtggtgtgagacgctcctgtctctcctctatctgcccatcggccctttggggaggaggaatgtgcccaaggactaaaaaaaggccatggagccagaggggcgagggcaacagacctttcatgggcaaaccttggggccctgctgtctagcatgccccactacgggtctaggctgcccatgtaaggaggcaaggcctggggacacccgagatgcctggttataattaacccagacatgtggctgcccccccccccccaacacctgctgcctctaaaaataaccctgtccctggtggatcccctgcatgcgaagatcttcgaacaaggctgtgggggactgagggcaggctgtaacaggcttgggggccagggcttatacgtgcctgggactcccaaagtattactgttccatgttcccggcgaagggccagctgtcccccgccagctagactcagcacttagtttaggaaccagtgagcaagtcagcccttggggcagcccatacaaggccatggggctgggcaagctgcacgcctgggtccggggtgggcacggtgcccgggcaacgagctgaaagctcatctgctctcaggggcccctccctggggacagcccctcctggctagtcacaccctgtaggctcctctatataacccaggggcacaggggctgccctcattctaccaccacctccacagcacagacagacactcaggagccagccagcc

SEQ ID NO: 34 - protein, 16 aa, Artificial Sequence
  QBEnd10-binding epitope
ELPTQGTFSNVSTNVS

SEQ ID NO: 35 - protein, 214 aa, Artificial Sequence
  SHP-1 SH2 complete domain
MVRWFHRDLSGLDAETLLKGRGVHGSFLARPSRKNQGDFSLSVRVGDQVTHIRIQNSGDFYDLYGGEKFATLTELVEYYTQQQGVLQDRDGTIIHLKYPLNCSDPTSERWYHGHMSGGQAETLLQAKGEPWTFLVRESLSQPGDFVLSVLSDQPKAGPGSPLRVTHIKVMCEGGRYTVGGLETFDSLTDLVEHFKKTGIEEASGAFVYLRQPYY

SEQ ID NO: 36 - protein, 97 aa, Artificial Sequence
  SHP-1 SH2 1 sequence
WFHRDLSGLDAETLLKGRGVHGSFLARPSRKNQGDFSLSVRVGDQVTHIRIQNSGDFYDLYGGEKFATLTELVEYYTQQQGVLQDRDGTIIHLKYPL

SEQ ID NO: 37 - protein, 104 aa, Artificial Sequence
  SHP-1 SH2 2 sequence
WYHGHMSGGQAETLLQAKGEPWTFLVRESLSQPGDFVLSVLSDQPKAGPGSPLRVTHIKVMCEGGRYTVGGLETFDSLTDLVEHFKKTGIEEASGAFVYLRQPY

SEQ ID NO: 38 - protein, 97 aa, Artificial Sequence
  SHP-2 first SH2 domain
WFHPNITGVEAENLLLTRGVDGSFLARPSKSNPGDFTLSVRRNGAVTHIKIQNTGDYYDLYGGEKFATLAELVQYYMEHHGQLKEKNGDVIELKYPL

SEQ ID NO: 39 - protein, 105 aa, Artificial Sequence
  SHP-2 second SH2 domain
WFHGHLSGKEAEKLLTEKGKHGSFLVRESQSHPGDFVLSVRTGDDKGESNDGKSKVTHVMIRCQELKYDVGGGERFDSLTDLVEHYKKNPMVETLGTVLQLKQPL

SEQ ID NO: 40 - protein, 211 aa, Artificial Sequence
  SHP-2 both SH2 domains
WFHPNITGVEAENLLLTRGVDGSFLARPSKSNPGDFTLSVRRNGAVTHIKIQNTGDYYDLYGGEKFATLAELVQYYMEHHGQLKEKNGDVIELKYPLNCADPTSERWFHGHLSGKEAEKLLTEKGKHGSFLVRESQSHPGDFVLSVRTGDDKGESNDGKSKVTHVMIRCQELKYDVGGGERFDSLTDLVEHYKKNPMVETLGTVLQLKQPL

SEQ ID NO: 41 - protein, 196 aa, Artificial Sequence
  truncated TGF beta receptor 2 sequence
MGWSCIILFLVATATGVHSTIPPHVQKSVNNDMIVTDNNGAVKFPQLCKFCDVRFSTCDNQKSCMSNCSITSICEKPQEVCVAVWRKNDENITLETVCHDPKLPYHDFILEDAASPKCIMKEKKKPGETFFMCSCSSDECNDNIIFSEEYNTSNPDLLLVIFQVTGISLLPPLGVAISVIIIFYCYRVNRQQKLSS

SEQ ID NO: 42 - protein, 517 aa, Artificial Sequence
  transgene FRB-FKBP12-L3-dCasp9
MASRILWHEMWHEGLEEASRLYFGERNVKGMFEVLEPLHAMMERGPQTLKETSFNQAYGRDLMEAQEWCRKYMKSGNVKDLLQAWDLYYHVFRRISKLEYSGGGSLEGVQVETISPGDGRTFPKRGQTCVVHYTGMLEDGKKFDSSRDRNKPFKFMLGKQEVIRGWEEGVAQMSVGQRAKLTISPDYAYGATGHPGIIPPHATLVFDVELLKLESGGGGSGGGGSGGGGSGVDGFGDVGALESLRGNADLAYILSMEPCGHCLIINNVNFCRESGLRTRTGSNIDCEKLRRRFSSLHFMVEVKGDLTAKKMVLALLELAQQDHGALDCCVVVILSHGCQASHLQFPGAVYGTDGCPVSVEKIVNIFNGTSCPSLGGKPKLFFIQACGGEQKDHGFEVASTSPEDESPGSNPEPDATPFQEGLRTFDQLDAISSLPTPSDIFVSYSTFPGFVSWRDPKSGSWYVETLDDIFEQWAHSEDLQSLLLRVANAVSVKGIYKQMPGCFNFLRKKLFFKTSAS

SEQ ID NO: 43 - protein, 136 aa, Artificial Sequence
  sort-suicide gene RQR8
CPYSNPSLCSGGGGSELPTQGTFSNVSTNVSPAKPTTTACPYSNPSLCSGGGGSPAPRPPTPAPTIASQPLSLRPEACRPAAGGAVHTRGLDFACDIYIWAPLAGTCGVLLLSLVITLYCNHRNRRRVCKCPRPVV

SEQ ID NO: 44 - protein, 20 aa, Foot-and-mouth disease virus
RAEGRGSLLTCGDVEENPGP

SEQ ID NO: 45 - protein, 20 aa, Foot-and-mouth disease virus
QCTNYALLKLAGDVESNPGP

SEQ ID NO: 46 - DNA, 17 bp, Artificial Sequence
  GAL4 DNA binding sequence
  misc_feature (4)..(14): n is a, c, g, or t
cggnnnnnnnnnnnccg

SEQ ID NO: 47 - DNA, 10 bp, Artificial Sequence
  Transcription factor C/EBP recognition sequence
attgcgcaat